European Patent Application EP 4 763 989 A1, published June 24, 2026. Title: ネコブセンチュウ及び葉かび病に抵抗性を有するトマト植物. Applicant: 株式会社サカタのタネ. The sequence listing filed with the application follows.

SEQUENCE LISTING (11 sequences)

SEQ ID NO: 1 - protein, 1257 aa, Solanum lycopersicum
MEKRKDIEEANNSLVLFSALSKDIANVLIFLENEENQKALDKDQVEKLKLKMAFICTYVQLSYSDFEQFEDIMTRNRQEVENLLQSLLDDDVLTSLTSNMDDCISLYHRSYKSDAIMMDEQLDFLLLNLYHLSKHHAEKIFPGVTQYEVLQNVCGNIRDFHGLILNGCIKHEMVENVLPLFQLMAERVGHFLWEDQTDEDSRLSELDEDEHNDRDSRLFQLTHLLLKIVPTELEVMHICYTNLKASTSAEVGRFIKKLLETSPDILREYIIQLQEHMLTVIPPSTLGARNIHVMMEFLLLILSDMPKDFIHHDKLFDLLAHVGTLTREVSTLVRDLEEKLRNKEGNNQTNCATLDLLENIELLKKDLKHVYLKAPNSSQCCFPMSDGPLFMHLLHMHLNDLLDSNAYSISLIKEEIELVSQELEFIRSFFGDAAEQGLYKDIWARVLDVAYEAKDVIDSIIVRDNGLLHLIFSLPITIKKIKLIKEEISALDENIPKDRGLIVVNSPKKPVERKSLTTDKIIVGFEEETNLILRKLTSGPADLDVISITGMPGSGKTTLAYKVYNDKSVSRHFDLRAWCTVDQGYDDKKLLDTIFSQVSGSDSNLSENIDVADKLRKQLFGKRYLIVLDDVWDTTTLDELTRPFPEAKKGSRIILTTREKEVALHGKLNTDPLDLRLLRPDESWELLDKRTFGNESCPDELLDVGKEIAENCKGLPLVADLIAGVIAGREKKRSVWLEVQSSLSSFILNSEVEVMKVIELSYDHLPHHLKPCLLHFASWPKDTPLTIYLFTVYLGAEGFVEKTEMKGIEEVVKIYMDDLISSSLVICFNEIGDILNFQIHDLVHDFCLIKARKENLFDRIRSSAPSDLLPRQITIDYDEEEEHFGLNFVMFDSNKKRHSGKHLYSLRINGDQLDDSVSDAFHLRHLRLIRVLDLEPSLIMVNDSLLNEICMLNHLRYLRIRTQVKYLPFSFSNLWNLESLFVSNKGSILVLLPRILDLVKLRVLSVGACSFFDMDADESILIAKDTKLENLRILGELLISYSKDTMNIFKRFPNLQVLQFELKESWDYSTEQHWFPKLDCLTELETLCVGFKSSNTNHCGSSVVTNRPWDFHFPSNLKELLLYDFPLTSDSLSTIARLPNLENLSLYDTIIQGEEWNMGEEDTFENLKFLNLRLLTLSKWEVGEESFPNLEKLKLQECGKLEEIPPSFGDIYSLKFIKIVKSPQLEDSALKIKKYAEDMRGGNDLQILGQKNIPLFK

SEQ ID NO: 2 - protein, 968 aa, Solanum lycopersicum
MMMVTSKVFSSLQFFTVFYLFTVAFASTEEATALLKWKATFKNQNNSFLASWTTSSNACKDWYGVVCLNGRVNTLNITNASVIGTLYAFPFSSLPFLENLDLSNNNISGTIPPEIGNLTNLVYLDLNTNQISGTIPPQIGSLAKLQIIRIFNNHLNGFIPEEIGYLRSLTKLSLGINFLSGSIPASLGNMTNLSFLFLYENQLSGFIPEEIGYLRSLTKLSLDINFLSGSIPASLGNLNNLSFLYLYNNQLSGSIPEEIGYLRSLTKLSLGINFLSGSIPASLGNLNNLSRLDLYNNKLSGSIPEEIGYLRSLTYLDLGENALNGSIPSSLGNLNNLSRLDLYNNKLSGSIPEEIGYLRSLTYLDLGENALNGSIPASLGNLNNLFMLYLYNNQLSGSIPEEIGYLSSLTELYLGNNSLNGSIPASLGNLNNLFMLYLYNNQLSGSIPEEIGYLSSLTELFLGNNSLNGSIPASLGNLNNLSRLYLYNNQLSGSIPASFGNMRNLQTLFLSDNDLIGEIPSFVCNLTSLEVLYMSRNNLKGKVPQCLGNISDLHILSMSSNSFRGELPSSISNLTSLKILDFGRNNLEGAIPQFFGNISSLQVFDMQNNKLSGTLPTNFSIGCSLISLNLHGNELADEIPRSLDNCKKLQVLDLGDNQLNDTFPMWLGTLPELRVLRLTSNKLHGPIRSSGAEIMFPDLRIIDLSRNAFSQDLPTSLFEHLKGMRTVDKTMEEPSYESYYDDSVVVVTKGLELEIVRILSLYTIIDLSSNKFEGHIPSVLGDLIAIRVLNVSHNALQGYIPSSLGSLSILESLDLSFNQLSGEIPQQLASLTFLEVLNLSHNYLQGCIPQGPQFRTFESNSYEGNDGLRGYPVSKGCGKDPVSEKNYTVSALEDQESNSEFFNDFWKAALMGYGSGLCIGISIIYILISTGNLRWLARIIEELEHKIIVQRRKKQRGQRNYRRRNNRF

SEQ ID NO: 3 - DNA, 24 bp, synthetic construct
  source 1..24: mol_type = other DNA
tggaaaaatgttgaatttcttttg

SEQ ID NO: 4 - DNA, 24 bp, synthetic construct
  source 1..24: mol_type = other DNA
gcatactatatggcttgtttaccc

SEQ ID NO: 5 - DNA, 46 bp, synthetic construct
  source 1..46: mol_type = other DNA
gaaggtgaccaagttcatgctgaagagaattagattgcactaaccc

SEQ ID NO: 6 - DNA, 46 bp, synthetic construct
  source 1..46: mol_type = other DNA
gaaggtcggagtcaacggattgaagagaattagattgcactaacca

SEQ ID NO: 7 - DNA, 21 bp, synthetic construct
  source 1..21: mol_type = other DNA
taaggcatcaaaggcgttaga

SEQ ID NO: 8 - DNA, 21 bp, synthetic construct
  source 1..21: mol_type = other DNA
agcagatgaaatccctcggtc

SEQ ID NO: 9 - DNA, 21 bp, synthetic construct
  source 1..21: mol_type = other DNA
cctcgctgcttctttctcctt

SEQ ID NO: 10 - RNA, 3982 nt, Solanum lycopersicum
  source 1..3982: mol_type = mRNA
  CDS 87..3860
tccaatagcttcaacattatttctcaaacaaagggttctctagctaaacttcagccagtgtaaaggtcttgagaaaaagtagaatcatggaaaaacgaaaagatattgaagaagcaaacaactcattggtgttattttctgctcttagcaaggacattgccaatgttctaattttcctagagaatgaggaaaatcaaaaagctcttgacaaagatcaagttgaaaagctaaaattgaaaatggcatttatttgtacatatgttcagctttcttattccgattttgagcagtttgaagatataatgactagaaatagacaagaggttgagaatctgcttcaatcacttttggatgatgatgtccttactagcctcaccagtaatatggatgactgtatcagcttgtatcatcgttcttataaatcagatgccatcatgatggatgagcaattggacttcctcctcttgaatctgtatcatctatccaagcatcacgctgaaaagatatttcctggagtgactcaatatgaagttcttcagaatgtatgtggcaacataagagatttccatgggttgatactgaatggttgcattaagcatgagatggttgagaatgtcttacctctgtttcaactcatggctgaaagagtaggacacttcctttgggaggatcagactgatgaagactctcggctctccgagctagatgaggatgaacacaatgatagagactctcgactcttccagctaacacatctactcttgaagattgttccaactgaactggaggttatgcacatatgttatacaaatttgaaagcttcaacttcagcagaagttggacgcttcattaagaagctcctggaaacctcaccggatattctcagagaatatatcattcaactacaagagcatatgttaactgttattccccctagcactttaggggctcgaaacattcatgtcatgatggaattcctattacttattctttctgatatgcccaaggactttattcatcatgacaaactttttgatctcttggctcatgttggaacacttaccagggaggtatcgactcttgtacgtgacttggaagagaaattaaggaataaagagggtaataaccaaacaaattgtgcaaccctagacttgctggaaaatattgaactcctcaagaaagatctcaaacatgtttatctgaaagccccaaattcatctcaatgttgcttccccatgagtgatggaccactcttcatgcatcttctacacatgcacttaaatgatttgctagattctaatgcttattcaatttctttgataaaggaagaaatcgagttggtgagtcaagaactggaattcataagatcattctttggggatgctgctgagcaaggattgtataaagatatctgggcacgtgttctagatgtggcttatgaggcaaaagatgtcatagattcaattattgttcgagataatggtctcttacatcttattttctcacttcccattaccataaagaagatcaaacttatcaaagaagagatctctgctttagatgagaacattcccaaggacagaggtctaatcgttgtgaactctcccaagaaaccagttgagagaaagtcattgacaactgataaaataattgtaggttttgaggaggagacaaacttgatacttagaaagctcaccagtggacccgcagatttagatgtcatttcgatcaccggtatgccgggttcaggtaaaactactttggcatacaaagtatacaatgataagtcagtttctagacattttgaccttcgtgcatggtgcacggtcgatcaaggatatgacgacaagaagttgttggatacaattttcagtcaagttagtggctcagattcaaatttgagtgagaatattgatgttgctgataaattgcggaaacaactgtttggaaagaggtatcttattgtcttagatgatgtgtgggatactactacattggatgagttgacaagaccttttcctgaagctaagaaaggaagtaggattattttgacaactcgagaaaaggaagtggctttgcatggaaagctgaacactgatcctcttgaccttcgattgctaagaccagatgaaagttgggaacttttagataaaaggacatttggtaatgagagttgccctgatgaactattagatgtcggtaaagaaatagccgaaaattgtaaagggcttcctttggtggctgatctgattgctggagtcattgctgggagggaaaagaaaaggagtgtgtggcttgaagttcaaagtagtttgagttcttttattttgaacagtgaagtggaagtgatgaaagttatagaattaagttatgaccatttaccacatcacctcaagccatgcttgcttcactttgcaagttggccgaaggacactcctttgacaatctatttgtttactgtttatttgggtgctgaaggatttgtggaaaagacggagatgaagggtatagaagaagtggtgaagatttatatggatgatttaatttccagtagcttggtaatttgtttcaatgagataggtgatatactgaatttccaaattcatgatcttgtgcatgacttttgtttgataaaagcaagaaaggaaaatttgtttgatcggataagatcaagtgctccatcagatttgttgcctcgtcaaattaccattgattatgatgaggaggaggagcactttgggcttaattttgtcatgttcgattcaaataagaaaaggcattctggtaaacacctctattctttgaggataaatggagaccagctggatgacagtgtttctgatgcatttcacctaagacacttgaggcttattagagtgttggacctggaaccctctttaatcatggtgaatgattctttgctgaatgaaatatgcatgttgaatcatttgaggtacttaagaattcggacacaagttaaatatctgcctttctctttctcaaacctctggaatctagaaagtctgtttgtgtctaacaaaggatcaatcttggtactattaccgagaattttggatcttgtaaagttgcgagtgctgtccgtgggtgcttgttctttctttgatatggatgcagatgaatcaatattgatagcaaaggacacaaagttagagaacttgagaatattaggggaactgttgatttcctattcgaaagatacaatgaatattttcaaaaggtttcccaatcttcaggtgcttcagtttgaactcaaggagtcatgggattattcaacagagcaacattggttcccgaaattggattgcctaactgaactagaaacactctgtgtaggttttaaaagttcaaacacaaaccactgtgggtcctctgttgtgacaaatcggccgtgggattttcacttcccttcaaatttgaaagaactgttgttgtatgactttcctctgacatccgattcactatcaacaatagcgagactgcccaaccttgaaaatttgtccctttatgatacaatcatccagggagaagaatggaacatgggggaggaagacacttttgagaatctcaaatttttgaacttgcgtctactgactctttccaagtgggaggttggagaggaatccttccccaatcttgagaaattaaaactgcaggaatgtggtaagcttgaggagattccacctagttttggagatatttattcattgaaatttatcaaaattgtaaagagtcctcaacttgaagattctgctctcaagattaagaaatacgctgaagatatgagaggagggaacgatcttcagatccttggccagaagaatatccccttatttaagtagcattttggttgaactttgcttggtgatattgtatatgattaaaatatcctgtgatgagattcctcttagtttcttttaacaaaaaatataatttttataagtacaaaaaaaaaaaaaaaaaa

SEQ ID NO: 11 - DNA, 3979 bp, Solanum lycopersicum
  source 1..3979: mol_type = genomic DNA
  CDS 654..3560
atcgattttagagtcattgcaatttaattttatcaaaatatttgagcatgaaaaatttgaaatggaggtgtcataaaaataaaataccctttacaacacgactttattgagttgacgatagttcaagtagggaaaataaataacttattatttgaatataaaacttgcaaaaaaaaaaaagtgatattcaaatttaattctgaccattatctcttgatattctttgctcttcatttatttgaatattcatttttcaaaagttccacatcataagacatcaaatatcaagtaggtcccataaaaataaaatacccttctcaacatgacaaagaaagattgaaaaatgactaacattttctcaaagacaaaaacaaaacatgtgagagaagagaattttgaaccaaatgtattatacactaagagtggtcatgatcattgtgtgataacaaaactattttggcaactttgactcagtccttggctaaattagacctctaacacaacagtccaaaagttgacttgagaatgacaacattttcttccctgatagcaaccaaattagcaaatttggaaaaaacgtgtgtcttgttgatctctaattagtataagtaacgtacaatatcctattgaatcggaaacaataaactcacactatgatgatggttactagcaaagtattctcttcacttcagtttttcactgttttctacctctttacagttgcatttgcttcgactgaggaggcaactgccctcttgaaatggaaagcaactttcaagaaccagaataattcctttttggcttcatggacgacaagttctaatgcatgcaaggactggtatggagttgtatgcttgaatggtagggtaaacacgttgaatattacaaatgccagtgtcattggtacactttatgcttttccattttcatccctcccttttctcgagaatcttgatcttagcaacaacaatatctctggtaccattccacctgagattggtaatctcacaaatcttgtctatcttgacttgaacaccaatcagatttcaggaacaattccaccacaaatcggttcactagccaagcttcagatcatccgcatatttaacaatcatttaaatggctttattcctgaagaaataggttacctaaggtctcttactaagctatctttgggtatcaactttcttagtggttctattcctgcttcattgggcaatatgaccaacttgtcttttttatttctttatgaaaatcagctttctggctttattcctgaagaaataggttacctaaggtctcttactaagctatctttggatatcaactttcttagtggttccattcctgcttcattggggaatctgaacaacttgtcttttttgtatctttacaataatcagctttctggctctattcctgaagaaataggttacctaaggtcacttactaagctatctttgggtatcaactttcttagtggttccattcctgcttcattggggaatctaaacaacttgtctaggttggatctttacaataataagctttctggctctattcctgaagaaataggttacctaaggtctcttacttacctagatttgggtgagaatgctcttaatggctctattccttcttcattggggaatctaaacaacttgtctaggttggatctttacaataataagctttctggctctattcctgaagaaataggttacctaaggtctcttacttacctagatttgggtgagaatgctcttaatggctctattcctgcttcattggggaatctgaacaacttgtttatgttgtatctttacaataatcagctttctggctctattcctgaagaaataggttacctgagttctcttactgaactatatttgggtaataactctcttaatggctctattcctgcttcattggggaatctgaacaacttgtttatgttgtatctttacaataatcagctttctggctctattcctgaagaaataggttacctgagttctcttactgaactatttttgggtaataactctcttaatggctctattcctgcttcattggggaatctaaacaacttgtctaggttgtatctttacaataatcagctttctggctctattcctgcttcatttggcaatatgagaaatctgcaaactctgtttctcagtgataacgatctcattggggaaattccttcatttgtgtgcaatttgacatcactggaagtgttgtatatgtcgagaaacaatttgaagggaaaagttccgcaatgtttgggtaatatcagtgaccttcacattttgtcgatgtcatctaatagtttcagaggagagctcccttcatctatttccaatttaacatcactaaaaatacttgattttggcagaaacaatctggagggagcaataccacaattttttggcaatattagtagcctccaggtttttgatatgcagaataacaaactttctgggactcttccaacaaattttagcattggatgttcactgataagtctcaacttgcatggcaatgaactagcagatgaaatccctcggtctttggacaattgcaaaaagctgcaagttcttgatttaggagacaatcaactcaacgacacatttcccatgtggttgggaactttgccagagctgagagttttaaggttgacatcgaataaattgcatggacctataagatcatcaggggctgaaatcatgtttcctgatctccgaatcatagatctctctcgcaatgcattctcgcaagacttaccaacgagtctatttgaacatttgaaagggatgaggacagttgataaaacaatggaggaaccaagttatgaaagctattacgatgactcggtggtagttgtgacaaagggattggagcttgaaattgtgagaattctgtctttgtacacaattatcgatctttcaagcaacaaatttgaaggacatattccttctgtcctgggagatctcattgcgatccgtgtacttaatgtatctcataatgcattgcaaggctatataccatcatcacttggaagtttatctatactggaatcactagacctttcgtttaaccaactttcgggagagataccacaacaacttgcttctcttacgtttcttgaagtcttaaatctctcccacaattatctccaaggatgcatccctcaaggacctcaattccgtacctttgagagcaattcatatgaaggtaatgatggattacgtggatatccagtttcaaaaggttgtggcaaagatcctgtgtcagagaaaaactatacagtgtctgcgctagaagatcaagaaagcaattctgaatttttcaatgatttttggaaagcagctctgatgggctatggaagtggactgtgtattggcatatccataatatatatcttgatctcgactggaaatctaagatggcttgcaagaatcattgaagaactggaacacaaaattatcgtgcaaaggagaaagaagcagcgaggtcaaagaaattacagaagaagaaataatcgcttctagacaagttaccaatacagaaagatttgatttcagaacttcaggtattcaagctaacctctaacacttatcttttttagtttattctaacaactaatatatgtttttttttttatcaacaaatacttattaacgcttgagacaaattgctagtaatcagttggaagttgtgatatataacaaaggctaaaaatttatagttgtgtgactcactttcttatttttccagattttcaggagccaagaataagaagacgctggtgtaaaggatttgcttcttcctgtgttgcagcttatgatgttggattagatttttagttttataagcttttcttcagttgggaaaatgtaatattatgaattttgatgatatacaataaatgttgtgtttattgaatgatatgtatgcatttatcggatcc